European Patent Application EP 4 442 701 A1, published October 9, 2024. Title: THE COMBINATION OF MOLECULAR SWITCH REGULATORY CHIMERIC ANTIGEN RECEPTOR CELLS AND ANTIBODIES AND USE THEREOF. Applicant: INNOVENT CELLS PHARMACEUTICALS (SU ZHOU) CO., LTD. The sequence listing filed with the application follows.

SEQUENCE LISTING (95 sequences)

SEQ ID NO: 1 - protein, 21 aa, artificial sequence
MALPVTALLLPLALLLHAARP

SEQ ID NO: 2 - protein, 119 aa, artificial sequence
EVQLVESGGGLVQPGGSLRLSCAASGFTFSRYWMNWVRQAPGKGLEWVGEITPDSSTINYAPSLKGRFTISRDNAKNSLYLQMNSLRAEDTAVYYCARPYDYGAWFASWGQGTLVTVSS

SEQ ID NO: 3 - protein, 109 aa, artificial sequence
QAVVTQEPSLTVSPGGTVTLTCRSSTGAVTTSNYANWVQEKPDHLFTGLIGGTNKRAPGTPARFSGSLLGGKAALTLSGAQPEDEAEYYCALWYSNHWVFGGGTKLTVL

SEQ ID NO: 4 - protein, 20 aa, artificial sequence
GGGGSGGGGSGGGGSGGGGS

SEQ ID NO: 5 - protein, 5 aa, artificial sequence
GGGGS

SEQ ID NO: 6 - protein, 12 aa, artificial sequence
ESKYGPPCPPCP

SEQ ID NO: 7 - protein, 39 aa, artificial sequence
IEVMYPPPYLDNEKSNGTIIHVKGKHLCPSPLFPGPSKP

SEQ ID NO: 8 - protein, 27 aa, artificial sequence
FWVLVVVGGVLACYSLLVTVAFIIFWV

SEQ ID NO: 9 - protein, 24 aa, artificial sequence
IYIWAPLAGTCGVLLLSLVITLYC

SEQ ID NO: 10 - protein, 41 aa, artificial sequence
RSKRSRLLHSDYMNMTPRRPGPTRKHYQPYAPPRDFAAYRS

SEQ ID NO: 11 - protein, 42 aa, artificial sequence
KRGRKKLLYIFKQPFMRPVQTTQEEDGCSCRFPEEEEGGCEL

SEQ ID NO: 12 - protein, 41 aa, artificial sequence
RSKRSRLLHSDYMFMTPRRPGPTRKHYQPYAPPRDFAAYRS

SEQ ID NO: 13 - protein, 112 aa, artificial sequence
RVKFSRSADAPAYQQGQNQLYNELNLGRREEYDVLDKRRGRDPEMGGKPRRKNPQEGLYNELQKDKMAEAYSEIGMKGERRRGKGHDGLYQGLSTATKDTYDALHMQALPPR

SEQ ID NO: 14 - protein, 55 aa, artificial sequence
KNRKAKAKPVTRGAGAGGRQRGQNKERPPPVPNPDYEPIRKGQRDLYSGLNQRRI

SEQ ID NO: 15 - protein, 303 aa, artificial sequence
MALPVTALLLPLALLLHAARPEVQLVESGGGLVQPGGSLRLSCAASGFTFSRYWMNWVRQAPGKGLEWVGEITPDSSTINYAPSLKGRFTISRDNAKNSLYLQMNSLRAEDTAVYYCARPYDYGAWFASWGQGTLVTVSSGGGGSGGGGSGGGGSGGGGSQAVVTQEPSLTVSPGGTVTLTCRSSTGAVTTSNYANWVQEKPDHLFTGLIGGTNKRAPGTPARFSGSLLGGKAALTLSGAQPEDEAEYYCALWYSNHWVFGGGTKLTVLGGGGSFWVLVVVGGVLACYSLLVTVAFIIFWVRS

SEQ ID NO: 16 - protein, 912 aa, artificial sequence
ATGGCCCTGCCTGTGACAGCACTGCTACTGCCTCTGGCTCTTCTGTTGCATGCTGCTAGACCTGAGGTTCAGTTGGTGGAGTCTGGGGGTGGATTAGTGCAGCCTGGGGGTAGTCTGAGACTGAGCTGTGCTGCCTCTGGCTTCACCTTCAGCAGATATTGGATGAACTGGGTGAGACAAGCCCCTGGCAAGGGCCTGGAGTGGGTGGGGGAGATCACCCCTGACAGCAGCACCATCAACTATGCCCCTAGCCTGAAGGGCAGATTCACCATCAGCAGAGACAATGCCAAGAACAGCCTGTACCTGCAGATGAACAGCCTGAGAGCTGAGGACACAGCTGTGTACTATTGTGCTAGACCCTATGACTATGGGGCCTGGTTTGCTAGCTGGGGCCAAGGCACCCTGGTAACAGTAAGCTCTGGGGGAGGGGGCTCTGGGGGGGGGGGGTCTGGGGGGGGGGGCTCTGGGGGGGGAGGCTCTCAAGCTGTGGTGACCCAAGAGCCTAGCCTCACTGTGAGCCCTGGGGGCACAGTGACCCTGACCTGCAGAAGCAGCACTGGGGCTGTGACCACAAGCAACTATGCCAACTGGGTGCAAGAGAAGCCTGACCACCTGTTTACTGGCCTGATTGGGGGCACCAACAAGAGAGCCCCTGGCACCCCTGCTAGATTTTCTGGCAGCCTCCTGGGGGGCAAGGCTGCCCTGACCCTGTCTGGGGCACAACCTGAGGATGAGGCTGAGTACTACTGTGCTCTCTGGTACAGCAACCACTGGGTGTTTGGGGGGGGCACCAAATTGACAGTGTTGGGTGGGGGGGGCTCCTTTTGGGTGCTGGTGGTGGTGGGGGGGGTGCTGGCCTGCTACAGCCTGTTAGTAACAGTGGCCTTTATCATCTTCTGGGTGAGAAGCTGA

SEQ ID NO: 17 - protein, 113 aa, artificial sequence
RVKFSRSADAPAYQQGQNQLYNELNLGRREEYDVLDKRRGRDPEMGGKPQRRKNPQEGLYNELQKDKMAEAYSEIGMKGERRRGKGHDGLYQGLSTATKDTYDALHMQALPPR

SEQ ID NO: 18 - protein, 45 aa, artificial sequence
TTTPAPRPPTPAPTIASQPLSLRPEACRPAAGGAVHTRGLDFACD

SEQ ID NO: 19-20 - skipped (2 entries)

SEQ ID NO: 21 - protein, 461 aa, artificial sequence
MALPVTALLLPLALLLHAARPEVQLVESGGGLVQPGGSLRLSCAASGFTFSRYWMNWVRQAPGKGLEWVGEITPDSSTINYAPSLKGRFTISRDNAKNSLYLQMNSLRAEDTAVYYCARPYDYGAWFASWGQGTLVTVSSGGGGSGGGGSGGGGSGGGGSQAVVTQEPSLTVSPGGTVTLTCRSSTGAVTTSNYANWVQEKPDHLFTGLIGGTNKRAPGTPARFSGSLLGGKAALTLSGAQPEDEAEYYCALWYSNHWVFGGGTKLTVLESKYGPPCPPCPFWVLVVVGGVLACYSLLVTVAFIIFWVRSKRSRLLHSDYMNMTPRRPGPTRKHYQPYAPPRDFAAYRSRVKFSRSADAPAYQQGQNQLYNELNLGRREEYDVLDKRRGRDPEMGGKPRRKNPQEGLYNELQKDKMAEAYSEIGMKGERRRGKGHDGLYQGLSTATKDTYDALHMQALPPR

SEQ ID NO: 22 - protein, 1386 aa, artificial sequence
ATGGCCCTGCCTGTGACAGCCCTATTACTGCCCCTGGCCCTTCTGTTACATGCTGCTAGACCTGAGGTTCAACTGGTGGAGTCTGGGGGGGGCCTAGTGCAGCCTGGGGGCAGCCTGAGACTGAGCTGTGCTGCCTCTGGCTTCACCTTCAGCAGATACTGGATGAACTGGGTGAGACAAGCCCCTGGCAAGGGCCTGGAGTGGGTGGGGGAGATCACCCCTGACAGCAGCACCATCAACTATGCCCCTAGCCTGAAGGGCAGATTCACCATCAGCAGAGACAATGCCAAGAACAGCCTGTACCTGCAGATGAACAGCCTGAGAGCTGAGGACACAGCTGTGTATTATTGTGCTAGACCATATGACTATGGGGCCTGGTTTGCCTCTTGGGGCCAAGGCACACTGGTTACAGTGAGTTCTGGGGGGGGGGGTTCTGGAGGGGGGGGATCTGGGGGTGGAGGTTCTGGGGGGGGGGGCAGTCAAGCTGTGGTGACCCAAGAGCCTAGCCTGACAGTGTCCCCTGGGGGCACAGTCACCCTGACCTGCAGAAGCAGCACTGGGGCTGTGACCACAAGCAACTATGCCAACTGGGTGCAAGAGAAGCCTGACCACCTGTTCACTGGCCTGATTGGGGGCACCAACAAAAGAGCCCCTGGCACCCCTGCTAGATTCTCTGGAAGCCTGTTGGGGGGCAAGGCTGCCCTGACCCTATCTGGGGCACAGCCTGAGGATGAGGCTGAGTACTACTGTGCCCTCTGGTACAGCAACCACTGGGTGTTTGGGGGGGGCACCAAACTGACAGTGTTGGAGAGCAAGTATGGCCCCCCCTGTCCTCCCTGTCCCTTTTGGGTGCTGGTGGTTGTGGGGGGGGTGCTGGCCTGCTACAGCCTGCTGGTGACAGTGGCCTTCATCATCTTCTGGGTGAGAAGCAAGAGAAGCAGACTGCTGCACTCTGACTACATGAACATGACCCCTAGAAGACCTGGCCCCACAAGAAAGCACTATCAGCCCTATGCCCCCCCTAGAGACTTTGCTGCCTACAGAAGCAGAGTGAAGTTCAGCAGATCTGCTGATGCCCCTGCCTATCAGCAAGGGCAGAATCAGCTGTATAATGAGCTCAACCTGGGCAGAAGAGAGGAGTATGATGTGCTGGACAAGAGAAGAGGCAGAGACCCTGAGATGGGGGGCAAGCCTAGAAGAAAGAACCCCCAAGAGGGCCTGTACAATGAGCTGCAAAAGGACAAGATGGCTGAGGCCTACTCTGAGATTGGCATGAAGGGGGAGAGAAGAAGAGGCAAGGGCCATGATGGCCTGTACCAAGGCCTGAGCACAGCCACCAAGGACACCTATGATGCCCTACATATGCAAGCTCTGCCCCCTAGATGA

SEQ ID NO: 23 - protein, 488 aa, artificial sequence
MALPVTALLLPLALLLHAARPEVQLVESGGGLVQPGGSLRLSCAASGFTFSRYWMNWVRQAPGKGLEWVGEITPDSSTINYAPSLKGRFTISRDNAKNSLYLQMNSLRAEDTAVYYCARPYDYGAWFASWGQGTLVTVSSGGGGSGGGGSGGGGSGGGGSQAVVTQEPSLTVSPGGTVTLTCRSSTGAVTTSNYANWVQEKPDHLFTGLIGGTNKRAPGTPARFSGSLLGGKAALTLSGAQPEDEAEYYCALWYSNHWVFGGGTKLTVLIEVMYPPPYLDNEKSNGTIIHVKGKHLCPSPLFPGPSKPFWVLVVVGGVLACYSLLVTVAFIIFWVRSKRSRLLHSDYMNMTPRRPGPTRKHYQPYAPPRDFAAYRSRVKFSRSADAPAYQQGQNQLYNELNLGRREEYDVLDKRRGRDPEMGGKPRRKNPQEGLYNELQKDKMAEAYSEIGMKGERRRGKGHDGLYQGLSTATKDTYDALHMQALPPR

SEQ ID NO: 24 - protein, 1467 aa, artificial sequence
ATGGCACTTCCTGTGACAGCCTTGTTACTACCTCTGGCCCTTCTTCTCCATGCTGCTAGACCTGAGGTGCAGCTGGTGGAGTCTGGGGGGGGCCTGGTACAACCTGGGGGCTCTCTGAGACTGAGCTGTGCTGCCTCTGGCTTCACCTTCAGCAGATATTGGATGAACTGGGTGAGACAAGCCCCTGGCAAGGGCCTGGAGTGGGTGGGGGAGATCACCCCTGACAGCAGCACCATCAACTATGCCCCTAGCCTGAAGGGCAGATTCACCATCAGCAGAGACAATGCCAAGAACAGCCTGTACCTGCAGATGAACAGCCTGAGAGCTGAGGACACAGCTGTGTACTATTGTGCTAGACCCTATGACTATGGGGCCTGGTTTGCTAGCTGGGGCCAAGGCACCCTTGTGACAGTCTCATCTGGGGGAGGGGGCAGTGGGGGGGGGGGCAGTGGGGGGGGGGGGTCTGGGGGAGGGGGGAGCCAAGCTGTGGTGACTCAAGAGCCAAGCCTGACAGTGAGCCCTGGGGGCACTGTGACCCTGACCTGCAGAAGCAGCACTGGGGCTGTGACCACAAGCAACTATGCCAACTGGGTGCAAGAGAAGCCTGACCACCTGTTTACTGGCCTGATTGGGGGCACCAATAAAAGAGCCCCTGGCACCCCTGCTAGATTCTCTGGCAGCCTCCTGGGGGGCAAGGCTGCCCTGACTCTGAGTGGGGCTCAGCCTGAGGATGAGGCTGAGTACTACTGTGCTCTCTGGTACAGCAACCACTGGGTGTTTGGGGGGGGCACCAAGCTTACAGTGCTGATTGAGGTGATGTACCCCCCCCCCTACCTGGACAATGAGAAAAGCAATGGCACCATCATCCATGTGAAGGGCAAGCACCTGTGCCCTAGCCCCCTGTTTCCTGGCCCTAGCAAACCCTTCTGGGTGCTAGTGGTGGTGGGGGGGGTGCTGGCCTGCTACAGCCTGTTAGTAACAGTGGCCTTTATCATCTTCTGGGTGAGAAGCAAGAGAAGCAGACTGCTGCACTCTGACTACATGAACATGACCCCTAGAAGACCTGGCCCCACAAGAAAGCACTATCAGCCCTATGCCCCCCCTAGAGACTTTGCTGCCTACAGAAGCAGAGTGAAGTTCAGCAGATCTGCTGATGCCCCTGCCTATCAGCAAGGGCAGAATCAGCTGTATAATGAGCTCAACCTGGGCAGAAGAGAGGAGTATGATGTGCTGGACAAGAGAAGAGGCAGAGACCCTGAGATGGGGGGCAAGCCTAGAAGAAAGAACCCCCAAGAGGGCCTGTACAATGAGCTGCAAAAGGACAAGATGGCTGAGGCCTACTCTGAGATTGGCATGAAGGGGGAGAGAAGAAGAGGCAAGGGCCATGATGGCCTGTACCAAGGCCTGAGCACAGCCACCAAGGACACCTATGATGCACTTCACATGCAAGCCCTGCCCCCTAGATGA

SEQ ID NO: 25 - protein, 452 aa, artificial sequence
MALPVTALLLPLALLLHAARPEVQLVESGGGLVQPGGSLRLSCAASGFTFSRYWMNWVRQAPGKGLEWVGEITPDSSTINYAPSLKGRFTISRDNAKNSLYLQMNSLRAEDTAVYYCARPYDYGAWFASWGQGTLVTVSSGGGGSGGGGSGGGGSGGGGSQAVVTQEPSLTVSPGGTVTLTCRSSTGAVTTSNYANWVQEKPDHLFTGLIGGTNKRAPGTPARFSGSLLGGKAALTLSGAQPEDEAEYYCALWYSNHWVFGGGTKLTVLGGGGSIYIWAPLAGTCGVLLLSLVITLYCKRGRKKLLYIFKQPFMRPVQTTQEEDGCSCRFPEEEEGGCELRVKFSRSADAPAYQQGQNQLYNELNLGRREEYDVLDKRRGRDPEMGGKPRRKNPQEGLYNELQKDKMAEAYSEIGMKGERRRGKGHDGLYQGLSTATKDTYDALHMQALPPR

SEQ ID NO: 26 - protein, 1359 aa, artificial sequence
ATGGCCCTGCCTGTGACAGCCCTACTACTGCCCCTGGCCCTTCTGCTTCATGCTGCTAGACCTGAGGTGCAGCTGGTGGAATCTGGGGGGGGCTTGGTTCAGCCTGGGGGCAGCCTGAGACTGAGCTGTGCTGCCTCTGGCTTCACCTTCAGCAGATATTGGATGAACTGGGTGAGACAAGCCCCTGGCAAGGGCCTGGAGTGGGTGGGGGAGATCACCCCTGACAGCAGCACCATCAACTATGCCCCTAGCCTGAAGGGCAGATTCACCATCAGCAGAGACAATGCCAAGAACAGCCTGTACCTGCAGATGAACAGCCTGAGAGCTGAGGACACAGCTGTGTACTATTGTGCTAGACCCTATGACTATGGGGCCTGGTTTGCTAGCTGGGGCCAAGGCACCCTAGTAACAGTGTCATCTGGGGGGGGAGGATCTGGGGGGGGGGGTTCTGGGGGGGGGGGCTCTGGTGGGGGGGGTTCTCAAGCTGTGGTAACACAAGAGCCTAGCCTGACAGTGAGCCCTGGGGGCACAGTGACCCTGACCTGCAGAAGCAGCACTGGGGCTGTGACCACAAGCAACTATGCCAACTGGGTGCAAGAGAAGCCTGACCACCTGTTCACTGGCCTGATTGGGGGCACCAATAAGAGAGCACCTGGCACTCCTGCTAGATTTTCTGGCTCACTGCTGGGGGGCAAGGCTGCCTTGACCCTTTCTGGGGCTCAGCCTGAGGATGAGGCTGAGTACTACTGTGCTCTCTGGTACAGCAACCACTGGGTGTTTGGGGGGGGCACCAAGCTGACAGTGCTGGGGGGGGGGGGTAGCATCTACATCTGGGCCCCCCTGGCTGGCACATGTGGGGTGCTGCTGCTGAGCCTGGTGATCACCCTGTACTGCAAGAGAGGCAGAAAGAAGCTGCTGTACATCTTCAAGCAGCCCTTCATGAGACCTGTGCAGACCACCCAAGAGGAGGATGGCTGCAGCTGCAGATTCCCTGAGGAGGAGGAGGGGGGCTGTGAGCTGAGAGTGAAGTTCAGCAGATCTGCTGATGCCCCTGCCTATCAGCAAGGGCAGAATCAGCTGTATAATGAGCTCAACCTGGGCAGAAGAGAGGAGTATGATGTGCTGGACAAGAGAAGAGGCAGAGACCCTGAGATGGGGGGCAAGCCTAGAAGAAAGAACCCCCAAGAGGGCCTGTACAATGAGCTGCAAAAGGACAAGATGGCTGAGGCCTACTCTGAGATTGGCATGAAGGGGGAGAGAAGAAGAGGCAAGGGCCATGATGGCCTGTACCAAGGCCTGAGCACAGCCACCAAGGACACTTATGATGCCTTGCACATGCAAGCCCTGCCTCCAAGATGA

SEQ ID NO: 27-30 - skipped (4 entries)

SEQ ID NO: 31 - protein, 494 aa, artificial sequence
MALPVTALLLPLALLLHAARPDIVMTQSPDSLAVSLGERATINCKSSQSLFNSGNQKNYLTWYQQKPGQPPKLLIYWASTRESGVPDRFSGSGSGTDFTLTISSLQAEDVAVYYCQNAYSFPYTFGGGTKLEIKRGGGGSGGGGSGGGGSQVQLQESGPGLIKPSQTLSLTCTVSGGSISSGYNWHWIRQPPGKGLEWIGYIHYTGSTNYNPALRSRVTISVDTSKNQFSLKLSSVTAADTAIYYCARIYNGNSFPYWGQGTTVTVSSTTTPAPRPPTPAPTIASQPLSLRPEACRPAAGGAVHTRGLDFACDFWVLVVVGGVLACYSLLVTVAFIIFWVRSKRSRLLHSDYMNMTPRRPGPTRKHYQPYAPPRDFAAYRSRVKFSRSADAPAYQQGQNQLYNELNLGRREEYDVLDKRRGRDPEMGGKPQRRKNPQEGLYNELQKDKMAEAYSEIGMKGERRRGKGHDGLYQGLSTATKDTYDALHMQALPPR

SEQ ID NO: 32 - protein, 393 aa, artificial sequence
MALPVTALLLPLALLLHAARPGMRTEDLPKAVVFLEPQWYRVLEKDSVTLKCQGAYSPEDNSTQWFHNESLISSQASSYFIDAATVDDSGEYRCQTNLSTLSDPVQLEVHIGWLLLQAPRWVFKEEDPIHLRCHSWKNTALHKVTYLQNGKGRKYFHHNSDFYIPKATLKDSGSYFCRGLVGSKNVSSETVNITITQGLAVSTISSFFPPGYQFWVLVVVGGVLACYSLLVTVAFIIFWVRSKRSRLLHSDYMNMTPRRPGPTRKHYQPYAPPRDFAAYRSRVKFSRSADAPAYQQGQNQLYNELNLGRREEYDVLDKRRGRDPEMGGKPRRKNPQEGLYNELQKDKMAEAYSEIGMKGERRRGKGHDGLYQGLSTATKDTYDALHMQALPPR

SEQ ID NO: 33 - protein, 493 aa, artificial sequence
MALPVTALLLPLALLLHAARPDIVLTQSPPSLAMSLGKRATISCRASESVTILGSHLIHWYQQKPGQPPTLLIQLASNVQTGVPARFSGSGSRTDFTLTIDPVEEDDVAVYYCLQSRTIPRTFGGGTKLEIKGSTSGSGKPGSGEGSTKGQIQLVQSGPELKKPGETVKISCKASGYTFTDYSINWVKRAPGKGLKWMGWINTETREPAYAYDFRGRFAFSLETSASTAYLQINNLKYEDTATYFCALDYSYAMDYWGQGTSVTVSSAAATTTPAPRPPTPAPTIASQPLSLRPEACRPAAGGAVHTRGLDFACDIYIWAPLAGTCGVLLLSLVITLYCKRGRKKLLYIFKQPFMRPVQTTQEEDGCSCRFPEEEEGGCELRVKFSRSADAPAYQQGQNQLYNELNLGRREEYDVLDKRRGRDPEMGGKPRRKNPQEGLYNELQKDKMAEAYSEIGMKGERRRGKGHDGLYQGLSTATKDTYDALHMQALPPR

SEQ ID NO: 34 - protein, 122 aa, artificial sequence
EVQLLDSGGGLVQPGGSLRLSCAASGFTFSSYVMSWVRQAPGKGLNWVSTISHSGGSTYYADSVKGRFTISRDNSKNTLYLQMNSLRAEDTAVYYCAIDAPYYDILTGYRYWGQGTLVTVSS

SEQ ID NO: 35 - protein, 107 aa, artificial sequence
DIQMTQSPSTLSASVGDRVTITCRASQSISSWLAWYQQKPGKAPKLLIYKASSLESGVPSRFSGSGSGTEFTLTISSLQPDDFATYYCQQYNSYSYTFGQGTKLEIK

SEQ ID NO: 36 - protein, 118 aa, artificial sequence
QVQLVQSGAEVKKPGSSVKVSCKASGYSFSSYNIHWVRQAPGQGLEWMGYIAPFQGDSRYNQKFKGRVTITADKSTSTAYMELSSLRSEDTAVYYCARLNRGNSLDYWGQGTLVTVSS

SEQ ID NO: 37 - protein, 113 aa, artificial sequence
DIVMTQSPDSLAVSLGERATINCKSSQSLFNSGNQRNYLTWYQQKPGQPPKLLIYWASTRESGVPDRFSGSGSGTDFTLTISSLQAEDVAVYYCQNNYIYPLTFGGGTKVEIK

SEQ ID NO: 38 - protein, 330 aa, artificial sequence [sequence omitted]

SEQ ID NO: 39 - protein, 330 aa, artificial sequence
ASTKGPSVFPLAPSSKSTSGGTAALGCLVKDYFPEPVTVSWNSGALTSGVHTFPAVLQSSGLYSLSSVVTVPSSSLGTQTYICNVNHKPSNTKVDKKVEPKSCDKTHTCPPCPAPELLGGPSVFLFPPKPKDTLMISRTPEVTCVVVDVSHEDPEVKFNWYVDGVEVHNAKTKPREEQYNSTYRVVSVLTVLHQDWLNGKEYKCKVSNKALGAPIEKTISKAKGQPREPQVYTLPPSRDELTKNQVSLTCLVKGFYPSDIAVEWESNGQPENNYKTTPPVLDSDGSFFLYSKLTVDKSRWQQGNVFSCSVMHEALHNHYTQKSLSLSPGK

SEQ ID NO: 40 - protein, 107 aa, artificial sequence [sequence omitted]

SEQ ID NO: 41 - protein, 666 aa, artificial sequence
EVQLLDSGGGLVQPGGSLRLSCAASGFTFSSYVMSWVRQAPGKGLNWVSTISHSGGSTYYADSVKGRFTISRDNSKNTLYLQMNSLRAEDTAVYYCAIDAPYYDILTGYRYWGQGTLVTVSSASTKGPSVFPLAPSSKSTSGGTAALGCLVKDYFPEPVTVSWNSGALTSGVHTFPAVLQSSGLYSLSSVVTVPSSSLGTQTYICNVNHKPSNTKVDKKVEPKSCDKTHTCPPCPAPELLGGPSVFLFPPKPKDTLMISRTPEVTCVVVDVSHEDPEVKFNWYVDGVEVHNAKTKPREEQYNSTYRVVSVLTVLHQDWLNGKEYKCKVSNKALPAPIEKTISKAKGQPREPQVYTLPPSRDELTKNQVSLTCLVKGFYPSDIAVEWESNGQPENNYKTTPPVLDSDGSFFLYSKLTVDKSRWQQGNVFSCSVMHEALHNHYTQKSLSLSPGKDIQMTQSPSTLSASVGDRVTITCRASQSISSWLAWYQQKPGKAPKLLIYKASSLESGVPSRFSGSGSGTEFTLTISSLQPDDFATYYCQQYNSYSYTFGQGTKLEIKRTVAAPSVFIFPPSDEQLKSGTASVVCLLNNFYPREAKVQWKVDNALQSGNSQESVTEQDSKDSTYSLSSTLTLSKADYEKHKVYACEVTHQGLSSPVTKSFNRGEC

SEQ ID NO: 42 - protein, 115 aa, artificial sequence
QVQLVQSGAEVKKPGASVKVSCKASGYSFTTYWMHWVRQAPGQGLEWMGLIDPSDSETRLNQKFKDRVTMTVDTSTSTVYMELSSLRSEDTAVYYCASNRWLLGWGQGTLVTVSS

SEQ ID NO: 43 - protein, 113 aa, artificial sequence
DIVMTQSPDSLAVSLGERATINCKSSQSLLNSGNQKNYLTWYQQKPGQPPKLLIYWASTRESGVPDRFSGSGSGTDFTLTISSLQAEDVAVYYCQNDYSYPLTFGQGTKLEIK

SEQ ID NO: 44 - protein, 118 aa, artificial sequence
QVQLVQSGAEVKKPGSSVKVSCKASGYSFSSYNIHWVRQAPGQGLEWMGYIAPFQGDARYNQKFKGRVTITADKSTSTAYMELSSLRSEDTAVYYCARLNRGQSLDYWGQGTLVTVSS

SEQ ID NO: 45 - protein, 113 aa, artificial sequence
DIVMTQSPDSLAVSLGERATINCKSSQSLFNAGNQRNYLTWYQQKPGQPPKLLIYWASTRESGVPDRFSGSGSGTDFTLTISSLQAEDVAVYYCQNNYIYPLTFGGGTKVEIK

SEQ ID NO: 46 - protein, 118 aa, artificial sequence
QVQLVQSGAEVKKPGSSVKVSCKASGYSFSSYNIHWVRQAPGQGLEWMGYIAPFQGDARYNQKFKGRVTITADKSTSTAYMELSSLRSEDTAVYYCARLNRGNALDYWGQGTLVTVSS

SEQ ID NO: 47 - protein, 113 aa, artificial sequence
DIVMTQSPDSLAVSLGERATINCKSSQSLFQSGNQRNYLTWYQQKPGQPPKLLIYWASTRESGVPDRFSGSGSGTDFTLTISSLQAEDVAVYYCQNNYIYPLTFGGGTKVEIK

SEQ ID NO: 48 - protein, 118 aa, artificial sequence
QVQLVQSGAEVKKPGSSVKVSCKASGYSFSSYNISWVRQAPGQGLEWMGYIAPFQGDARYNQKFKGRVTITADKSTSTAYMELSSLRSEDTAVYYCARLNRGNSLDYWGQGTLVTVSS

SEQ ID NO: 49 - protein, 113 aa, artificial sequence; identical to SEQ ID NO: 37

SEQ ID NO: 50 - protein, 118 aa, artificial sequence
QVQLQQPGAELVRPGASVKLSCKASGYTFTSYWINWVKQRPGQGLEWIGNIYPSDSYTNYNQKFKDKATLTVDKSSSTAYMQLSSPTSEDSAVYYCTRSWRGNSFDYWGQGTTLTVSS

SEQ ID NO: 51 - protein, 113 aa, artificial sequence
DIQMTQSPSSLTVTAGEKVTMSCKSSQSLLNSGNQRNYLTWYQQIPGQPPKLLIYWSSTRGSGVPDRFTGSGSGTDFTLTISSVQAEDLAVYFCQNVYYYPFTFGSGTRLEVK

SEQ ID NO: 52 - protein, 477 aa, artificial sequence
EVQLVESGGGLVQPGGSLRLSCAASGFTFSRYWMNWVRQAPGKGLEWVGEITPDSSTINYAPSLKGRFTISRDNAKNSLYLQMNSLRAEDTAVYYCARPYDYGAWFASWGQGTLVTVSSGGGGSGGGGSGGGGSGGGGSQAVVTQEPSLTVSPGGTVTLTCRSSTGAVTTSNYANWVQEKPDHLFTGLIGGTNKRAPGTPARFSGSLLGGKAALTLSGAQPEDEAEYYCALWYSNHWVFGGGTKLTVLESKYGPPCPPCPAPELLGGPSVFLFPPKPKDTLMISRTPEVTCVVVDVSHEDPEVKFNWYVDGVEVHNAKTKPREEQYNSTYRVVSVLTVLHQDWLNGKEYKCKVSNKALPAPIEKTISKAKGQPREPQVYTLPPSRDELTKNQVSLTCLVKGFYPSDIAVEWESNGQPENNYKTTPPVLDSDGSFFLYSKLTVDKSRWQQGNVFSCSVMHEALHNHYTQKSLSLSPGK

SEQ ID NO: 53 - protein, 175 aa, artificial sequence
MALPVTALLLPLALLLHAARPAPELLGGPSVFLFPPKPKDTLMISRTPEVTCVVVDVSHEDPEVKFNWYVDGVEVHNAKTKPREEQYNSTYRVVSVLTVLHQDWLNGKEYKCKVSNKALGAPIEKTISKAKGGGGSGGGGSGGGGSGGGGSIYIWAPLAGTCGVLLLSLVITLYC

SEQ ID NO: 54 - protein, 5 aa, artificial sequence
RYWMN

SEQ ID NO: 55 - protein, 17 aa, artificial sequence
EITPDSSTINYAPSLKG

SEQ ID NO: 56 - protein, 10 aa, artificial sequence
PYDYGAWFAS

SEQ ID NO: 57 - protein, 14 aa, artificial sequence
RSSTGAVTTSNYAN

SEQ ID NO: 58 - protein, 7 aa, artificial sequence
GTNKRAP

SEQ ID NO: 59 - protein, 9 aa, artificial sequence
ALWYSNHWV

SEQ ID NO: 60 - protein, 5 aa, artificial sequence
SYVMS

SEQ ID NO: 61 - protein, 17 aa, artificial sequence
TISHSGGSTYYADSVKG

SEQ ID NO: 62 - protein, 13 aa, artificial sequence
DAPYYDILTGYRY

SEQ ID NO: 63 - protein, 11 aa, artificial sequence
RASQSISSWLA

SEQ ID NO: 64 - protein, 7 aa, artificial sequence
KASSLES

SEQ ID NO: 65 - protein, 9 aa, artificial sequence
QQYNSYSYT

SEQ ID NO: 66 - protein, 5 aa, artificial sequence
SYNIH

SEQ ID NO: 67 - protein, 17 aa, artificial sequence
YIAPFQGDSRYNQKFKG

SEQ ID NO: 68 - protein, 9 aa, artificial sequence
LNRGNSLDY

SEQ ID NO: 69 - protein, 17 aa, artificial sequence
KSSQSLFNSGNQRNYLT

SEQ ID NO: 70 - protein, 7 aa, artificial sequence
WASTRES

SEQ ID NO: 71 - protein, 9 aa, artificial sequence
QNNYIYPLT

SEQ ID NO: 72 - protein, 5 aa, artificial sequence
SYNIH

SEQ ID NO: 73 - protein, 17 aa, artificial sequence
YIAPFQGDARYNQKFKG

SEQ ID NO: 74 - protein, 9 aa, artificial sequence
LNRGQSLDY

SEQ ID NO: 75 - protein, 17 aa, artificial sequence
KSSQSLFNAGNQRNYLT

SEQ ID NO: 76 - protein, 7 aa, artificial sequence
WASTRES

SEQ ID NO: 77 - protein, 9 aa, artificial sequence
QNNYIYPLT

SEQ ID NO: 78 - protein, 5 aa, artificial sequence
SYNIH

SEQ ID NO: 79 - protein, 17 aa, artificial sequence
YIAPFQGDARYNQKFKG

SEQ ID NO: 80 - protein, 9 aa, artificial sequence
LNRGNALDY

SEQ ID NO: 81 - protein, 17 aa, artificial sequence
KSSQSLFQSGNQRNYLT

SEQ ID NO: 82 - protein, 7 aa, artificial sequence
WASTRES

SEQ ID NO: 83 - protein, 9 aa, artificial sequence
QNNYIYPLT

SEQ ID NO: 84 - protein, 5 aa, artificial sequence
SYNIS

SEQ ID NO: 85 - protein, 17 aa, artificial sequence
YIAPFQGDARYNQKFKG

SEQ ID NO: 86 - protein, 9 aa, artificial sequence
LNRGNSLDY

SEQ ID NO: 87 - protein, 17 aa, artificial sequence
KSSQSLFNSGNQRNYLT

SEQ ID NO: 88 - protein, 7 aa, artificial sequence
WASTRES

SEQ ID NO: 89 - protein, 9 aa, artificial sequence
QNNYIYPLT

SEQ ID NO: 90 - protein, 5 aa, artificial sequence
TYWMH

SEQ ID NO: 91 - protein, 17 aa, artificial sequence
LIDPSDSETRLNQKFKD

SEQ ID NO: 92 - protein, 6 aa, artificial sequence
NRWLLG

SEQ ID NO: 93 - protein, 17 aa, artificial sequence
KSSQSLLNSGNQKNYLT

SEQ ID NO: 94 - protein, 7 aa, artificial sequence
WASTRES

SEQ ID NO: 95 - protein, 9 aa, artificial sequence
QNDYSYPLT